European Patent Specification EP 3 885 369 B1, published October 9, 2024. Title: RECOMBINANT DEAMIDATED GLIADIN POLYPEPTIDE ANTIGEN, RECOMBINANT ANTIGEN-EXPRESSING GENE, RECOMBINANT EXPRESSION VECTOR, AND PREPARATION METHOD AND APPLICATION THEREOF. Applicant: SHENZHEN YHLO BIOTECH CO., LTD. The sequence listing filed with the application follows.

SEQUENCE LISTING (8 sequences)

SEQ ID NO: 1 - protein, 9 aa, Homo sapiens
PLQPEQPFP

SEQ ID NO: 2 - protein, 9 aa, Homo sapiens
PEQLPQFEE

SEQ ID NO: 3 - protein, 114 aa, Homo sapiens
NWVNVISDLKKIEDLIQSMHIDATLYTESDVHPSCKVTAMKCFLLELQVISLESGDASIHDTVENLIILANNSLSSNGNVTESGCKECEELEEKNIKEFLQSFVHIVQMFINTS

SEQ ID NO: 4 - protein, 6 aa, Artificial Sequence
HHHHHH

SEQ ID NO: 5 - protein, 7 aa, Artificial Sequence
DYKDDDK

SEQ ID NO: 6 - protein, 4 aa, Artificial Sequence
GSGS

SEQ ID NO: 7 - protein, 161 aa, Artificial Sequence
HHHHHHGSGSPLQPEQPFPGSGSNWVNVISDLKKIEDLIQSMHIDATLYTESDVHPSCKVTAMKCFLLELQVISLESGDASIHDTVENLIILANNSLSSNGNVTESGCKECEELEEKNIKEFLQSFVHIVQMFINTSGSGSPEQLPQFEEGSGSDYKDDDK

SEQ ID NO: 8 - DNA, 498 bp, Artificial Sequence
catatgcatcatcatcatcaccatggcagtggtagtccgctgcagccggaacagccgtttccgggcagtggcagcaattgggttaatgtgattagcgatctgaaaaagattgaagatctgattcagagtatgcatattgatgccaccctgtataccgaaagtgatgttcatccgagctgcaaagtgaccgccatgaaatgctttctgctggaactgcaggttattagcctggaaagcggtgacgccagtattcatgataccgtggaaaatctgattattctggccaataatagcctgagtagtaatggtaatgtgaccgaaagcggttgcaaagaatgcgaagaactggaagaaaagaatattaaggaattcctgcagagttttgttcatattgttcagatgtttatcaacaccagcggtagtggcagcccggaacagctgccgcagtttgaagaaggtagtggcagtgattataaagatgatgataaataaaagctt